European Patent Application EP 4 501 312 A1, published February 5, 2025. Title: Liquid formulation pharmaceutical composition comprising plasmid DNA. Applicant: Helixmith Co., Ltd. The sequence listing filed with the application follows.

SEQUENCE LISTING (22 sequences)

SEQ ID NO: 1 - protein, 728 aa, synthetic construct
MWVTKLLPALLLQHVLLHLLLLPIAIPYAEGQRKRRNTIHEFKKSAKTTLIKIDPALKIKTKKVNTADQCANRCTRNKGLPFTCKAFVFDKARKQCLWFPFNSMSSGVKKEFGHEFDLYENKDYIRNCIIGKGRSYKGTVSITKSGIKCQPWSSMIPHEHSFLPSSYRGKDLQENYCRNPRGEEGGPWCFTSNPEVRYEVCDIPQCSEVECMTCNGESYRGLMDHTESGKICQRWDHQTPHRHKFLPERYPDKGFDDNYCRNPDGQPRPWCYTLDPHTRWEYCAIKTCADNTMNDTDVPLETTECIQGQGEGYRGTVNTIWNGIPCQRWDSQYPHEHDMTPENFKCKDLRENYCRNPDGSESPWCFTTDPNIRVGYCSQIPNCDMSHGQDCYRGNGKNYMGNLSQTRSGLTCSMWDKNMEDLHRHIFWEPDASKLNENYCRNPDDDAHGPWCYTGNPLIPWDYCPISRCEGDTTPTIVNLDHPVISCAKTKQLRVVNGIPTRTNIGWMVSLRYRNKHICGGSLIKESWVLTARQCFPSRDLKDYEAWLGIHDVHGRGDEKCKQVLNVSQLVYGPEGSDLVLMKLARPAVLDDFVSTIDLPNYGCTIPEKTSCSVYGWGYTGLINYDGLLRVAHLYIMGNEKCSQHHRGKVTLNESEICAGAEKIGSGPCEGDYGGPLVCEQHKMRMVLGVIVPGRGCAIPNRPGIFVRVAYYAKWIHKIILTYKVPQS

SEQ ID NO: 2 - protein, 723 aa, synthetic construct
MWVTKLLPALLLQHVLLHLLLLPIAIPYAEGQRKRRNTIHEFKKSAKTTLIKIDPALKIKTKKVNTADQCANRCTRNKGLPFTCKAFVFDKARKQCLWFPFNSMSSGVKKEFGHEFDLYENKDYIRNCIIGKGRSYKGTVSITKSGIKCQPWSSMIPHEHSYRGKDLQENYCRNPRGEEGGPWCFTSNPEVRYEVCDIPQCSEVECMTCNGESYRGLMDHTESGKICQRWDHQTPHRHKFLPERYPDKGFDDNYCRNPDGQPRPWCYTLDPHTRWEYCAIKTCADNTMNDTDVPLETTECIQGQGEGYRGTVNTIWNGIPCQRWDSQYPHEHDMTPENFKCKDLRENYCRNPDGSESPWCFTTDPNIRVGYCSQIPNCDMSHGQDCYRGNGKNYMGNLSQTRSGLTCSMWDKNMEDLHRHIFWEPDASKLNENYCRNPDDDAHGPWCYTGNPLIPWDYCPISRCEGDTTPTIVNLDHPVISCAKTKQLRVVNGIPTRTNIGWMVSLRYRNKHICGGSLIKESWVLTARQCFPSRDLKDYEAWLGIHDVHGRGDEKCKQVLNVSQLVYGPEGSDLVLMKLARPAVLDDFVSTIDLPNYGCTIPEKTSCSVYGWGYTGLINYDGLLRVAHLYIMGNEKCSQHHRGKVTLNESEICAGAEKIGSGPCEGDYGGPLVCEQHKMRMVLGVIVPGRGCAIPNRPGIFVRVAYYAKWIHKIILTYKVPQS

SEQ ID NO: 3 - DNA, 482 bp, synthetic construct
  source 1..482: mol_type = other DNA
atgtgggtgaccaaactcctgccagccctgctgctgcagcatgtcctcctgcatctcctcctgctccccatcgccatcccctatgcagagggacaaaggaaaagaagaaatacaattcatgaattcaaaaaatcagcaaagactaccctaatcaaaatagatccagcactgaagataaaaaccaaaaaagtgaatactgcagaccaatgtgctaatagatgtactaggaataaaggacttccattcacttgcaaggcttttgtttttgataaagcaagaaaacaatgcctctggttccccttcaatagcatgtcaagtggagtgaaaaaagaatttggccatgaatttgacctctatgaaaacaaagactacattagaaactgcatcattggtaaaggacgcagctacaagggaacagtatctatcactaagagtggcatcaaatgtcagccctggagttccatgataccacacgaacacag

SEQ ID NO: 4 - DNA, 1675 bp, synthetic construct
  source 1..1675: mol_type = other DNA
cctacaggaaaactactgtcgaaatcctcgaggggaagaagggggaccctggtgtttcacaagcaatccagaggtacgctacgaagtctgtgacattcctcagtgttcagaagttgaatgcatgacctgcaatggggagagttatcgaggtctcatggatcatacagaatcaggcaagatttgtcagcgctgggatcatcagacaccacaccggcacaaattcttgcctgaaagatatcccgacaagggctttgatgataattattgccgcaatcccgatggccagccgaggccatggtgctatactcttgaccctcacacccgctgggagtactgtgcaattaaaacatgcgctgacaatactatgaatgacactgatgttcctttggaaacaactgaatgcatccaaggtcaaggagaaggctacaggggcactgtcaataccatttggaatggaattccatgtcagcgttgggattctcagtatcctcacgagcatgacatgactcctgaaaatttcaagtgcaaggacctacgagaaaattactgccgaaatccagatgggtctgaatcaccctggtgttttaccactgatccaaacatccgagttggctactgctcccaaattccaaactgtgatatgtcacatggacaagattgttatcgtgggaatggcaaaaattatatgggcaacttatcccaaacaagatctggactaacatgttcaatgtgggacaagaacatggaagacttacatcgtcatatcttctgggaaccagatgcaagtaagctgaatgagaattactgccgaaatccagatgatgatgctcatggaccctggtgctacacgggaaatccactcattccttgggattattgccctatttctcgttgtgaaggtgataccacacctacaatagtcaatttagaccatcccgtaatatcttgtgccaaaacgaaacaattgcgagttgtaaatgggattccaacacgaacaaacataggatggatggttagtttgagatacagaaataaacatatctgcggaggatcattgataaaggagagttgggttcttactgcacgacagtgtttcccttctcgagacttgaaagattatgaagcttggcttggaattcatgatgtccacggaagaggagatgagaaatgcaaacaggttctcaatgtttcccagctggtatatggccctgaaggatcagatctggttttaatgaagcttgccaggcctgctgtcctggatgattttgttagtacgattgatttacctaattatggatgcacaattcctgaaaagaccagttgcagtgtttatggctggggctacactggattgatcaactatgatggcctattacgagtggcacatctctatataatgggaaatgagaaatgcagccagcatcatcgagggaaggtgactctgaatgagtctgaaatatgtgctggggctgaaaagattggatcaggaccatgtgagggggattatggtggcccacttgtttgtgagcaacataaaatgagaatggttcttggtgtcattgttcctggtcgtggatgtgccattccaaatcgtcctggtatttttgtccgagtagcatattatgcaaaatggatacacaaaattattttaacatataaggtaccacagtcatag

SEQ ID NO: 5 - DNA, 4956 bp, synthetic construct
  source 1..4956: mol_type = other DNA
gtaagaacagtatgaagaaaagagatgaagcctctgtcttttttacatgttaacagtctcatattagtccttcagaataattctacaatcctaaaataacttagccaacttgctgaattgtattacggcaaggtttatatgaattcatgactgatatttagcaaatgattaattaatatgttaataaaatgtagccaaaacaatatcttaccttaatgcctcaatttgtagatctcggtatttgtgaaataataacgtaaacttcgtttaaaaggattcttcttcctgtctttgagaaagtacggcactgtgcagggggagaggttgattgtgaaaaatcagaggtagatgagaatcttactgagggctgagggttctttaaccttggtggatctcaacattggttgcacattaaaatcacctgctgcaagcccttgacgaatcttacttagaagatgacaacacagaacaattaaatcagaatctctggggagaatagggcaccagtattttttgagctcccaccatgattccaaagtgcagccaaatttgagaaccactgctaaaagctcaagcttcagattgaccagcttttccatctcacctatcgcctaaagaccaaattggataaatgtgttcattacgacagatgggtactatttaaagatgagtaaacacaatatacttaggctcgtcagactgagagttttaatcatcactgaggaaaaacatagatatctaatactgactggagtattagtcaaggcttatttcacacacaattttatcagaaaccaaagtagtttaaaacagctctccccttattagtaatgcattggagggtttactttaccatgtaccttgctgagcactgtaccttgttaatctcatttacttgtaatgagaaccacacagcgggtagttttattggttctattttacctacatgacaaaactgaagcataaaaacacttagtaagttttcagtgtcatgcacaactaggaagtgacatggccagaatataagcccagtcaccatcactctataacctgcgcttttaacaacttcagggcatgacacatttggccggtcagtagaacccatgctgtgatttgtttttgcagtggtggtgatgactgccttgttgaatccactttttattctattccattttggggacacaattctgcaagatgattcttcattaggaaacagagatgagttattgaccaacacagaaagaaaaagagtttgttgctccacactgggattaaacctatgatcttggcctaattaacactagctagtaagtgtccaagctgatcatctctacaacatttcaataacagaaaacaacaattttcaaaattagttacttacaattatgtagaaatgcctctaaaacacagtattttccttatattacaaaaacaaaaattataattggttttgtcctcttttgagagtttgcatggtgttactccctgcatagtgaagaaaacattttatttaagtagatggatctaagtttttcatgaacaaaggaatgacatttgaaatcaatcctaccctagtccaggagaatgcattagattaacctagtagaggtcttatttcaccctgagttttctatgatcgtgattctctgctggaggagtaattgtgaaatagatctctctgggaactggcttcctagtccaatcagctcttttaccaatgaacacttccttgtgatatagatgtttatggccgagaggatccagtatattaataaaatccctttttgtattcaatgagggaaacacataattttcatcaattagcagcttattggaatatctgcatgatggtttaacacttttaagtgttgactaaagattaattttacagaaaatagaaaaagaaatatgtttctgtctggaggaatgatttattgttgacccctaaattgaaatattttactagtggcttaatggaaagatgatgaaagatgatgaaattaatgtagaagcttaactagaaaatcaggtgacctgatatctacatctgtatccttcattggccacccagcattcattaatgaatcagatgatggaatagatcaagtttcctaggaacacagtgaatattaaaagaaaacaaagggagcctagcacctagaagacctagtttatatttcaaagtatatttggatgtaacccaattttaaacatttcctcacttgtctctcttaaagccttgccaacagcaaggacagagaaccaaaaatagtgtatatatgaataaatgcttattacagaatctgctgactggcacatgctttgtgtgtaatgggttctcataaacacttgttgaatgaacacacataagtgaaagagcatggctaggcttcatcccttggtcaaatatggggtgctaaagaaaagcaggggaaatacattgggacactaacaaaaaaaaacagttaatttaggtaaaagataaaatacaccacagaatgaagaaaagagatgacccagactgctctttaaccttcatgtcctagagaggtttttgatatgaattgcattcagaattgtggaaaggagcccatcttttctcttcattttgattttattaactccaatgggggaattttattcgtgttttggccatatctacttttgatttctacattattctctcttcctttctacctgtatttgtcctaataaattgttgacttattaattcactacttcctcacagcttttttttggctttacaaatccactggaaaggtatatgggtgtatcactttgtgtatttcggtgtgcatgtgtagaggggacaaaaatcctctctcaaactataaatattgagtatttgtgtattgaacatttgctataactactaggtttcttaaataatcttaatatataaaatgatatagaaaaagggaaattatagttcgtattattcatctaagtgaagagattaaaacccagggagtaaataaattgtctaaggactaaggttgtatactatttaggtgatagatatggggcaaccgtatgggttttatgattaacaaataaacttctcaccactctaccatatcaacttttccataaaagagagctatagtattctttgcttaaataaatttgattagtgcatgacttcttgaaaacatataaagcaaaagtcacatttgattctatcagaaaagtgagtaagccatggcccaaacaaaagatgcattaaaatattctggaatgatggagctaaaagtaagaaaaatgactttttaaaaaagtttactgttaggaattgtgaaattatgctgaattttagttgcattataatttttgtcagtcatacggtctgacaacctgtcttatttctatttccccatatgaggaatgctagttaagtatggatattaactattactacttagatgcattgaagttgcataatatggataatacttcactggttccctgaaaatgtttagttagtaataagtctcttacactatttgttttgtccaataatttatattttctgaagacttaactctagaatacactcatgtcaaaatgaaagaatttcattgcaaaatattgcttggtacatgacgcatacctgtatttgttttgtgtcacaacatgaaaaatgatggtttattagaagtttcattgggtaggaaacacatttgaatggtatttactaagatactaaaatccttggacttcactctaattttagtgccatttagaactcaaggtctcagtaaaagtagaaataaagcctgttaacaaaacacaaactgaatattaaaaatgtaactggattttcaaagaaatgtttactggtattacctgtagatgtatattctttattatgatcttttgtgtaaagtctggcagacaaatgcaatatctaattgttgagtccaatatcacaagcagtacaaaagtataaaaaagacttggccttttctaatgtgttaaaatactttatgctggtaataacactaagagtagggcactagaaattttaagtgaagataatgtgttgcagttactgcactcaatggcttactattataaaccaaaactgggatcactaagctccagtcagtcaaaatgatcaaaattattgaagagaataagcaattctgttctttattaggacacagtagatacagactacaaagtggagtgtgcttaataagaggtagcatttgttaagtgtcaattactctattatcccttggagcttctcaaaataaccatataaggtgtaagatgttaaaggttatggttacactcagtgcacaggtaagctaataggctgagagaagctaaattacttactggggtctcacagtaagaaagtgagctgaagtttcagcccagatttaactggattctgggctctttattcatgttacttcatgaatctgtttctcaattgtgcagaaaaaagggggctatttataagaaaagcaataaacaaacaagtaatgatctcaaataagtaatgcaagaaatagtgagatttcaaaatcagtggcagcgatttctcagttctgtcctaagtggccttgctcaatcacctgctatcttttagtggagctttgaaattatgtttcagacaacttcgattcagttctagaatgtttgactcagcaaattcacaggctcatctttctaacttgatggtgaatatggaaattcagctaaatggatgttaataaaattcaaacgttttaaggacagatggaaatgacagaattttaaggtaaaatatatgaaggaatataagataaaggatttttctaccttcagcaaaaacatacccactaattagtaaaattaataggcgaaaaaaagttgcatgctcttatactgtaatgattatcattttaaaactagctttttgccttcgagctatcggggtaaaga

SEQ ID NO: 6 - DNA, 3756 bp, synthetic construct
  source 1..3756: mol_type = other DNA
cgcgttgacattgattattgactagttattaatagtaatcaattacggggtcattagttcatagcccatatatggagttccgcgttacataacttacggtaaatggcccgcctggctgaccgcccaacgacccccgcccattgacgtcaataatgacgtatgttcccatagtaacgccaatagggactttccattgacgtcaatgggtggagtatttacggtaaactgcccacttggcagtacatcaagtgtatcatatgccaagtccgccccctattgacgtcaatgacggtaaatggcccgcctggcattatgcccagtacatgaccttacgggactttcctacttggcagtacatctacgtattagtcatcgctattaccatggtgatgcggttttggcagtacaccaatgggcgtggatagcggtttgactcacggggatttccaagtctccaccccattgacgtcaatgggagtttgttttggcaccaaaatcaacgggactttccaaaatgtcgtaataaccccgccccgttgacgcaaatgggcggtaggcgtgtacggtgggaggtctatataagcagagctcgtttagtgaaccgtcagatcgcctggagacgccatccacgctgttttgacctccatagaagacaccgggaccgatccagcctccgcggccgggaacggtgcattggaacgcggattccccgtgccaagagtgacgtaagtaccgcctatagactctataggcacacccctttggctcttatgcatgctatactgtttttggcttggggcctatacacccccgcttccttatgctataggtgatggtatagcttagcctataggtgtgggttattgaccattattgaccactcccctattggtgacgatactttccattactaatccataacatggctctttgccacaactatctctattggctatatgccaatactctgtccttcagagactgacacggactctgtatttttacaggatggggtcccatttattatttacaaattcacatatacaacaacgccgtcccccgtgcccgcagtttttattaaacatagcgtgggatctccacgcgaatctcgggtacgtgttccggacatgggctcttctccggtagcggcggagcttccacatccgagccctggtcccatgcctccagcggctcatggtcgctcggcagctccttgctcctaacagtggaggccagacttaggcacagcacaatgcccaccaccaccagtgtgccgcacaaggccgtggcggtagggtatgtgtctgaaaatgagctcggagattgggctcgcaccgctgacgcagatggaagacttaaggcagcggcagaagaagatgcaggcagctgagttgttgtattctgataagagtcagaggtaactcccgttgcggtgctgttaacggtggagggcagtgtagtctgagcagtactcgttgctgccgcgcgcgccaccagacataatagctgacagactaacagactgttcctttccatgggtcttttctgcagtcaccgtccttgacacgaagcttggtaccgagctcggatccactagtccagtgtggtggaattctgcagatatccagcacagtggcggccgctcgagtctagagggcccgtttaaacccgctgatcagcctcgactgtgccttctagttgccagccatctgttgtttgcccctcccccgtgccttccttgaccctggaaggtgccactcccactgtcctttcctaataaaatgaggaaattgcatcgcattgtctgagtaggtgtcattctattctggggggtggggtggggcaggacagcaagggggaggattgggaagacaatagcaggcatgctggggagtcgaaattcagaagaactcgtcaagaaggcgatagaaggcgatgcgctgcgaatcgggagcggcgataccgtaaagcacgaggaagcggtcagcccattcgccgccaagctcttcagcaatatcacgggtagccaacgctatgtcctgatagcggtccgccacacccagccggccacagtcgatgaatccagaaaagcggccattttccaccatgatattcggcaagcaggcatcgccatgggtcacgacgagatcctcgccgtcgggcatgctcgccttgagcctggcgaacagttcggctggcgcgagcccctgatgctcttcgtccagatcatcctgatcgacaagaccggcttccatccgagtacgtgctcgctcgatgcgatgtttcgcttggtggtcgaatgggcaggtagccggatcaagcgtatgcagccgccgcattgcatcagccatgatggatactttctcggcaggagcaaggtgagatgacaggagatcctgccccggcacttcgcccaatagcagccagtcccttcccgcttcagtgacaacgtcgagcacagctgcgcaaggaacgcccgtcgtggccagccacgatagccgcgctgcctcgtcttgcagttcattcagggcaccggacaggtcggtcttgacaaaaagaaccgggcgcccctgcgctgacagccggaacacggcggcatcagagcagccgattgtctgttgtgcccagtcatagccgaatagcctctccacccaagcggccggagaacctgcgtgcaatccatcttgttcaatcatgcgaaacgatcctcatcctgtctcttgatcagatcttgatcccctgcgccatcagatccttggcggcaagaaagccatccagtttactttgcagggcttcccaaccttaccagagggcgccccagctggcaattccggttcgcttgctgtccataaaaccgcccagtctagctatcgccatgtaagcccactgcaagctacctgctttctctttgcgcttgcgttttcccttgtccagatagcccagtagctgacattcatccggggtcagcaccgtttctgcggactggctttctacgtgaaaaggatctaggtgaagatcctttttgataatctcatgaccaaaatcccttaacgtgagttttcgttccactgagcgtcagaccccgtagaaaagatcaaaggatcttcttgagatcctttttttctgcgcgtaatctgctgcttgcaaacaaaaaaaccaccgctaccagcggtggtttgtttgccggatcaagagctaccaactctttttccgaaggtaactggcttcagcagagcgcagataccaaatactgttcttctagtgtagccgtagttaggccaccacttcaagaactctgtagcaccgcctacatacctcgctctgctaatcctgttaccagtggctgctgccagtggcgataagtcgtgtcttaccgggttggactcaagacgatagttaccggataaggcgcagcggtcgggctgaacggggggttcgtgcacacagcccagcttggagcgaacgacctacaccgaactgagatacctacagcgtgagctatgagaaagcgccacgcttcccgaagggagaaaggcggacaggtatccggtaagcggcagggtcggaacaggagagcgcacgagggagcttccagggggaaacgcctggtatctttatagtcctgtcgggtttcgccacctctgacttgagcgtcgatttttgtgatgctcgtcaggggggcggagcctatggaaaaacgccagcaacgcggcctttttacggttcctggccttttgctggccttttgctcacatg

SEQ ID NO: 7 - DNA, 7113 bp, synthetic construct
  source 1..7113: mol_type = other DNA
atgtgggtgaccaaactcctgccagccctgctgctgcagcatgtcctcctgcatctcctcctgctccccatcgccatcccctatgcagagggacaaaggaaaagaagaaatacaattcatgaattcaaaaaatcagcaaagactaccctaatcaaaatagatccagcactgaagataaaaaccaaaaaagtgaatactgcagaccaatgtgctaatagatgtactaggaataaaggacttccattcacttgcaaggcttttgtttttgataaagcaagaaaacaatgcctctggttccccttcaatagcatgtcaagtggagtgaaaaaagaatttggccatgaatttgacctctatgaaaacaaagactacattagaaactgcatcattggtaaaggacgcagctacaagggaacagtatctatcactaagagtggcatcaaatgtcagccctggagttccatgataccacacgaacacaggtaagaacagtatgaagaaaagagatgaagcctctgtcttttttacatgttaacagtctcatattagtccttcagaataattctacaatcctaaaataacttagccaacttgctgaattgtattacggcaaggtttatatgaattcatgactgatatttagcaaatgattaattaatatgttaataaaatgtagccaaaacaatatcttaccttaatgcctcaatttgtagatctcggtatttgtgaaataataacgtaaacttcgtttaaaaggattcttcttcctgtctttgagaaagtacggcactgtgcagggggagaggttgattgtgaaaaatcagaggtagatgagaatcttactgagggctgagggttctttaaccttggtggatctcaacattggttgcacattaaaatcacctgctgcaagcccttgacgaatcttacttagaagatgacaacacagaacaattaaatcagaatctctggggagaatagggcaccagtattttttgagctcccaccatgattccaaagtgcagccaaatttgagaaccactgctaaaagctcaagcttcagattgaccagcttttccatctcacctatcgcctaaagaccaaattggataaatgtgttcattacgacagatgggtactatttaaagatgagtaaacacaatatacttaggctcgtcagactgagagttttaatcatcactgaggaaaaacatagatatctaatactgactggagtattagtcaaggcttatttcacacacaattttatcagaaaccaaagtagtttaaaacagctctccccttattagtaatgcattggagggtttactttaccatgtaccttgctgagcactgtaccttgttaatctcatttacttgtaatgagaaccacacagcgggtagttttattggttctattttacctacatgacaaaactgaagcataaaaacacttagtaagttttcagtgtcatgcacaactaggaagtgacatggccagaatataagcccagtcaccatcactctataacctgcgcttttaacaacttcagggcatgacacatttggccggtcagtagaacccatgctgtgatttgtttttgcagtggtggtgatgactgccttgttgaatccactttttattctattccattttggggacacaattctgcaagatgattcttcattaggaaacagagatgagttattgaccaacacagaaagaaaaagagtttgttgctccacactgggattaaacctatgatcttggcctaattaacactagctagtaagtgtccaagctgatcatctctacaacatttcaataacagaaaacaacaattttcaaaattagttacttacaattatgtagaaatgcctctaaaacacagtattttccttatattacaaaaacaaaaattataattggttttgtcctcttttgagagtttgcatggtgttactccctgcatagtgaagaaaacattttatttaagtagatggatctaagtttttcatgaacaaaggaatgacatttgaaatcaatcctaccctagtccaggagaatgcattagattaacctagtagaggtcttatttcaccctgagttttctatgatcgtgattctctgctggaggagtaattgtgaaatagatctctctgggaactggcttcctagtccaatcagctcttttaccaatgaacacttccttgtgatatagatgtttatggccgagaggatccagtatattaataaaatccctttttgtattcaatgagggaaacacataattttcatcaattagcagcttattggaatatctgcatgatggtttaacacttttaagtgttgactaaagattaattttacagaaaatagaaaaagaaatatgtttctgtctggaggaatgatttattgttgacccctaaattgaaatattttactagtggcttaatggaaagatgatgaaagatgatgaaattaatgtagaagcttaactagaaaatcaggtgacctgatatctacatctgtatccttcattggccacccagcattcattaatgaatcagatgatggaatagatcaagtttcctaggaacacagtgaatattaaaagaaaacaaagggagcctagcacctagaagacctagtttatatttcaaagtatatttggatgtaacccaattttaaacatttcctcacttgtctctcttaaagccttgccaacagcaaggacagagaaccaaaaatagtgtatatatgaataaatgcttattacagaatctgctgactggcacatgctttgtgtgtaatgggttctcataaacacttgttgaatgaacacacataagtgaaagagcatggctaggcttcatcccttggtcaaatatggggtgctaaagaaaagcaggggaaatacattgggacactaacaaaaaaaaacagttaatttaggtaaaagataaaatacaccacagaatgaagaaaagagatgacccagactgctctttaaccttcatgtcctagagaggtttttgatatgaattgcattcagaattgtggaaaggagcccatcttttctcttcattttgattttattaactccaatgggggaattttattcgtgttttggccatatctacttttgatttctacattattctctcttcctttctacctgtatttgtcctaataaattgttgacttattaattcactacttcctcacagcttttttttggctttacaaatccactggaaaggtatatgggtgtatcactttgtgtatttcggtgtgcatgtgtagaggggacaaaaatcctctctcaaactataaatattgagtatttgtgtattgaacatttgctataactactaggtttcttaaataatcttaatatataaaatgatatagaaaaagggaaattatagttcgtattattcatctaagtgaagagattaaaacccagggagtaaataaattgtctaaggactaaggttgtatactatttaggtgatagatatggggcaaccgtatgggttttatgattaacaaataaacttctcaccactctaccatatcaacttttccataaaagagagctatagtattctttgcttaaataaatttgattagtgcatgacttcttgaaaacatataaagcaaaagtcacatttgattctatcagaaaagtgagtaagccatggcccaaacaaaagatgcattaaaatattctggaatgatggagctaaaagtaagaaaaatgactttttaaaaaagtttactgttaggaattgtgaaattatgctgaattttagttgcattataatttttgtcagtcatacggtctgacaacctgtcttatttctatttccccatatgaggaatgctagttaagtatggatattaactattactacttagatgcattgaagttgcataatatggataatacttcactggttccctgaaaatgtttagttagtaataagtctcttacactatttgttttgtccaataatttatattttctgaagacttaactctagaatacactcatgtcaaaatgaaagaatttcattgcaaaatattgcttggtacatgacgcatacctgtatttgttttgtgtcacaacatgaaaaatgatggtttattagaagtttcattgggtaggaaacacatttgaatggtatttactaagatactaaaatccttggacttcactctaattttagtgccatttagaactcaaggtctcagtaaaagtagaaataaagcctgttaacaaaacacaaactgaatattaaaaatgtaactggattttcaaagaaatgtttactggtattacctgtagatgtatattctttattatgatcttttgtgtaaagtctggcagacaaatgcaatatctaattgttgagtccaatatcacaagcagtacaaaagtataaaaaagacttggccttttctaatgtgttaaaatactttatgctggtaataacactaagagtagggcactagaaattttaagtgaagataatgtgttgcagttactgcactcaatggcttactattataaaccaaaactgggatcactaagctccagtcagtcaaaatgatcaaaattattgaagagaataagcaattctgttctttattaggacacagtagatacagactacaaagtggagtgtgcttaataagaggtagcatttgttaagtgtcaattactctattatcccttggagcttctcaaaataaccatataaggtgtaagatgttaaaggttatggttacactcagtgcacaggtaagctaataggctgagagaagctaaattacttactggggtctcacagtaagaaagtgagctgaagtttcagcccagatttaactggattctgggctctttattcatgttacttcatgaatctgtttctcaattgtgcagaaaaaagggggctatttataagaaaagcaataaacaaacaagtaatgatctcaaataagtaatgcaagaaatagtgagatttcaaaatcagtggcagcgatttctcagttctgtcctaagtggccttgctcaatcacctgctatcttttagtggagctttgaaattatgtttcagacaacttcgattcagttctagaatgtttgactcagcaaattcacaggctcatctttctaacttgatggtgaatatggaaattcagctaaatggatgttaataaaattcaaacgttttaaggacagatggaaatgacagaattttaaggtaaaatatatgaaggaatataagataaaggatttttctaccttcagcaaaaacatacccactaattagtaaaattaataggcgaaaaaaagttgcatgctcttatactgtaatgattatcattttaaaactagctttttgccttcgagctatcggggtaaagacctacaggaaaactactgtcgaaatcctcgaggggaagaagggggaccctggtgtttcacaagcaatccagaggtacgctacgaagtctgtgacattcctcagtgttcagaagttgaatgcatgacctgcaatggggagagttatcgaggtctcatggatcatacagaatcaggcaagatttgtcagcgctgggatcatcagacaccacaccggcacaaattcttgcctgaaagatatcccgacaagggctttgatgataattattgccgcaatcccgatggccagccgaggccatggtgctatactcttgaccctcacacccgctgggagtactgtgcaattaaaacatgcgctgacaatactatgaatgacactgatgttcctttggaaacaactgaatgcatccaaggtcaaggagaaggctacaggggcactgtcaataccatttggaatggaattccatgtcagcgttgggattctcagtatcctcacgagcatgacatgactcctgaaaatttcaagtgcaaggacctacgagaaaattactgccgaaatccagatgggtctgaatcaccctggtgttttaccactgatccaaacatccgagttggctactgctcccaaattccaaactgtgatatgtcacatggacaagattgttatcgtgggaatggcaaaaattatatgggcaacttatcccaaacaagatctggactaacatgttcaatgtgggacaagaacatggaagacttacatcgtcatatcttctgggaaccagatgcaagtaagctgaatgagaattactgccgaaatccagatgatgatgctcatggaccctggtgctacacgggaaatccactcattccttgggattattgccctatttctcgttgtgaaggtgataccacacctacaatagtcaatttagaccatcccgtaatatcttgtgccaaaacgaaacaattgcgagttgtaaatgggattccaacacgaacaaacataggatggatggttagtttgagatacagaaataaacatatctgcggaggatcattgataaaggagagttgggttcttactgcacgacagtgtttcccttctcgagacttgaaagattatgaagcttggcttggaattcatgatgtccacggaagaggagatgagaaatgcaaacaggttctcaatgtttcccagctggtatatggccctgaaggatcagatctggttttaatgaagcttgccaggcctgctgtcctggatgattttgttagtacgattgatttacctaattatggatgcacaattcctgaaaagaccagttgcagtgtttatggctggggctacactggattgatcaactatgatggcctattacgagtggcacatctctatataatgggaaatgagaaatgcagccagcatcatcgagggaaggtgactctgaatgagtctgaaatatgtgctggggctgaaaagattggatcaggaccatgtgagggggattatggtggcccacttgtttgtgagcaacataaaatgagaatggttcttggtgtcattgttcctggtcgtggatgtgccattccaaatcgtcctggtatttttgtccgagtagcatattatgcaaaatggatacacaaaattattttaacatataaggtaccacagtcatag

SEQ ID NO: 8 - DNA, 6190 bp, synthetic construct
  source 1..6190: mol_type = other DNA
atgtgggtgaccaaactcctgccagccctgctgctgcagcatgtcctcctgcatctcctcctgctccccatcgccatcccctatgcagagggacaaaggaaaagaagaaatacaattcatgaattcaaaaaatcagcaaagactaccctaatcaaaatagatccagcactgaagataaaaaccaaaaaagtgaatactgcagaccaatgtgctaatagatgtactaggaataaaggacttccattcacttgcaaggcttttgtttttgataaagcaagaaaacaatgcctctggttccccttcaatagcatgtcaagtggagtgaaaaaagaatttggccatgaatttgacctctatgaaaacaaagactacattagaaactgcatcattggtaaaggacgcagctacaagggaacagtatctatcactaagagtggcatcaaatgtcagccctggagttccatgataccacacgaacacaggtaagaacagtatgaagaaaagagatgaagcctctgtcttttttacatgttaacagtctcatattagtccttcagaataattctacaatcctaaaataacttagccaacttgctgaattgtattacggcaaggtttatatgaattcatgactgatatttagcaaatgattaattaatatgttaataaaatgtagccaaaacaatatcttaccttaatgcctcaatttgtagatctcggtatttgtgaaataataacgtaaacttcgtttaaaaggattcttcttcctgtctttgagaaagtacggcactgtgcagggggagaggttgattgtgaaaaatcagaggtagatgagaatcttactgagggctgagggttctttaaccttggtggatctcaacattggttgcacattaaaatcacctgctgcaagcccttgacgaatcttacttagaagatgacaacacagaacaattaaatcagaatctctggggagaatagggcaccagtattttttgagctcccaccatgattccaaagtgcagccaaatttgagaaccactgctaaaagctcaagcttcagattgaccagcttttccatctcacctatcgcctaaagaccaaattggataaatgtgttcattacgacagatgggtactatttaaagatgagtaaacacaatatacttaggctcgtcagactgagagttttaatcatcactgaggaaaaacatagatatctaatactgactggagtattagtcaaggcttatttcacacacaattttatcagaaaccaaagtagtttaaaacagctctccccttattagtaatgcattggagggtttactttaccatgtaccttgctgagcactgtaccttgttaatctcatttacttgtaatgagaaccacacagcgggtagttttattggttctattttacctacatgacaaaactgaagcataaaaacacttagtaagttttcagtgtcatgcacaactaggaagtgacatggccagaatataagcccagtcaccatcactctataacctgcgcttttaacaacttcagggcatgacacatttggccggtcagtagaacccatgctgtgatttgtttttgcagtggtggtgatgactgccttgttgaatccactttttattctattccattttggggacacaattctgcaagatgattcttcattaggaaacagagatgagttattgaccaacacagaaagaaaaagagtttgttgctccacactgggattaaacctatgatcttggcctaattaacactagctagtaagtgtccaagctgatcatctctacaacatttcaataacagaaaacaacaattttcaaaattagttacttacaattatgtagaaatgcctctaaaacacagtattttccttatattacaaaaacaaaaattataattggttttgtcctcttttgagagtttgcatggtgttactccctgcatagtgaagaaaacattttatttaagtagatggatctaagtttttcatgaacaaaggaatgacatttgaaatcaatcctaccctagtccaggagaatgcattagattaacctagtagaggtcttatttcaccctgagttttctatgatcgtgattctctgctggaggagtaattgtgaaatagatctctctgggaactggcttcctagtccaatcagctcttttaccaatgaacacttccttgtgatatagatgtttatggccgagaggatctcttcctttctacctgtatttgtcctaataaattgttgacttattaattcactacttcctcacagcttttttttggctttacaaatccactggaaaggtatatgggtgtatcactttgtgtatttcggtgtgcatgtgtagaggggacaaaaatcctctctcaaactataaatattgagtatttgtgtattgaacatttgctataactactaggtttcttaaataatcttaatatataaaatgatatagaaaaagggaaattatagttcgtattattcatctaagtgaagagattaaaacccagggagtaaataaattgtctaaggactaaggttgtatactatttaggtgatagatatggggcaaccgtatgggttttatgattaacaaataaacttctcaccactctaccatatcaacttttccataaaagagagctatagtattctttgcttaaataaatttgattagtgcatgacttcttgaaaacatataaagcaaaagtcacatttgattctatcagaaaagtgagtaagccatggcccaaacaaaagatgcattaaaatattctggaatgatggagctaaaagtaagaaaaatgactttttaaaaaagtttactgttaggaattgtgaaattatgctgaattttagttgcattataatttttgtcagtcatacggtctgacaacctgtcttatttctatttccccatatgaggaatgctagttaagtatggatattaactattactacttagatgcattgaagttgcataatatggataatacttcactggttccctgaaaatgtttagttagtaataagtctcttacactatttgttttgtccaataatttatattttctgaagacttaactctagaatacactcatgtcaaaatgaaagaatttcattgcaaaatattgcttggtacatgacgcatacctgtatttgttttgtgtcacaacatgaaaaatgatggtttattagaagtttcattgggtaggaaacacatttgaatggtatttactaagatactaaaatccttggacttcactctaattttagtgccatttagaactcaaggtctcagtaaaagtagaaataaagcctgttaacaaaacacaaactgaatattaaaaatgtaactggattttcaaagaaatgtttactggtattacctgtagatgtatattctttattatgatcttttgtgtaaagtctggcagacaaatgcaatatctaattgttgagtccaatatcacaagcagtacaaaagtataaaaaagacttggccttttctaatgtgttaaaatactttatgctggtaataacactaagagtagggcactagaaattttaagtgaagataatgtgttgcagttactgcactcaatggcttactattataaaccaaaactgggatcactaagctccagtcagtcaaaatgatcaaaattattgaagagaataagcaattctgttctttattaggacacagtagatacagactacaaagtggagtgtgcttaataagaggtagcatttgttaagtgtcaattactctattatcccttggagcttctcaaaataaccatataaggtgtaagatgttaaaggttatggttacactcagtgcacaggtaagctaataggctgagagaagctaaattacttactggggtctcacagtaagaaagtgagctgaagtttcagcccagatttaactggattctgggctctttattcatgttacttcatgaatctgtttctcaattgtgcagaaaaaagggggctatttataagaaaagcaataaacaaacaagtaatgatctcaaataagtaatgcaagaaatagtgagatttcaaaatcagtggcagcgatttctcagttctgtcctaagtggccttgctcaatcacctgctatcttttagtggagctttgaaattatgtttcagacaacttcgattcagttctagaatgtttgactcagcaaattcacaggctcatctttctaacttgatggtgaatatggaaattcagctaaatggatgttaataaaattcaaacgttttaaggacagatggaaatgacagaattttaaggtaaaatatatgaaggaatataagataaaggatttttctaccttcagcaaaaacatacccactaattagtaaaattaataggcgaaaaaaagttgcatgctcttatactgtaatgattatcattttaaaactagctttttgccttcgagctatcggggtaaagacctacaggaaaactactgtcgaaatcctcgaggggaagaagggggaccctggtgtttcacaagcaatccagaggtacgctacgaagtctgtgacattcctcagtgttcagaagttgaatgcatgacctgcaatggggagagttatcgaggtctcatggatcatacagaatcaggcaagatttgtcagcgctgggatcatcagacaccacaccggcacaaattcttgcctgaaagatatcccgacaagggctttgatgataattattgccgcaatcccgatggccagccgaggccatggtgctatactcttgaccctcacacccgctgggagtactgtgcaattaaaacatgcgctgacaatactatgaatgacactgatgttcctttggaaacaactgaatgcatccaaggtcaaggagaaggctacaggggcactgtcaataccatttggaatggaattccatgtcagcgttgggattctcagtatcctcacgagcatgacatgactcctgaaaatttcaagtgcaaggacctacgagaaaattactgccgaaatccagatgggtctgaatcaccctggtgttttaccactgatccaaacatccgagttggctactgctcccaaattccaaactgtgatatgtcacatggacaagattgttatcgtgggaatggcaaaaattatatgggcaacttatcccaaacaagatctggactaacatgttcaatgtgggacaagaacatggaagacttacatcgtcatatcttctgggaaccagatgcaagtaagctgaatgagaattactgccgaaatccagatgatgatgctcatggaccctggtgctacacgggaaatccactcattccttgggattattgccctatttctcgttgtgaaggtgataccacacctacaatagtcaatttagaccatcccgtaatatcttgtgccaaaacgaaacaattgcgagttgtaaatgggattccaacacgaacaaacataggatggatggttagtttgagatacagaaataaacatatctgcggaggatcattgataaaggagagttgggttcttactgcacgacagtgtttcccttctcgagacttgaaagattatgaagcttggcttggaattcatgatgtccacggaagaggagatgagaaatgcaaacaggttctcaatgtttcccagctggtatatggccctgaaggatcagatctggttttaatgaagcttgccaggcctgctgtcctggatgattttgttagtacgattgatttacctaattatggatgcacaattcctgaaaagaccagttgcagtgtttatggctggggctacactggattgatcaactatgatggcctattacgagtggcacatctctatataatgggaaatgagaaatgcagccagcatcatcgagggaaggtgactctgaatgagtctgaaatatgtgctggggctgaaaagattggatcaggaccatgtgagggggattatggtggcccacttgtttgtgagcaacataaaatgagaatggttcttggtgtcattgttcctggtcgtggatgtgccattccaaatcgtcctggtatttttgtccgagtagcatattatgcaaaatggatacacaaaattattttaacatataaggtaccacagtcatag

SEQ ID NO: 9 - DNA, 5190 bp, synthetic construct
  source 1..5190: mol_type = other DNA
atgtgggtgaccaaactcctgccagccctgctgctgcagcatgtcctcctgcatctcctcctgctccccatcgccatcccctatgcagagggacaaaggaaaagaagaaatacaattcatgaattcaaaaaatcagcaaagactaccctaatcaaaatagatccagcactgaagataaaaaccaaaaaagtgaatactgcagaccaatgtgctaatagatgtactaggaataaaggacttccattcacttgcaaggcttttgtttttgataaagcaagaaaacaatgcctctggttccccttcaatagcatgtcaagtggagtgaaaaaagaatttggccatgaatttgacctctatgaaaacaaagactacattagaaactgcatcattggtaaaggacgcagctacaagggaacagtatctatcactaagagtggcatcaaatgtcagccctggagttccatgataccacacgaacacaggtaagaacagtatgaagaaaagagatgaagcctctgtcttttttacatgttaacagtctcatattagtccttcagaataattctacaatcctaaaataacttagccaacttgctgaattgtattacggcaaggtttatatgaattcatgactgatatttagcaaatgattaattaatatgttaataaaatgtagccaaaacaatatcttaccttaatgcctcaatttgtagatctcggtatttgtgaaataataacgtaaacttcgtttaaaaggattcttcttcctgtctttgagaaagtacggcactgtgcagggggagaggttgattgtgaaaaatcagaggtagatgagaatcttactgagggctgagggttctttaaccttggtggatctcaacattggttgcacattaaaatcacctgctgcaagcccttgacgaatcttacttagaagatgacaacacagaacaattaaatcagaatctctggggagaatagggcaccagtattttttgagctcccaccatgattccaaagtgcagccaaatttgagaaccactgctaaaagctcaagcttcagattgaccagcttttccatctcacctatcgcctaaagaccaaattggataaatgtgttcattacgacagatgggtactatttaaagatgagtaaacacaatatacttaggctcgtcagactgagagttttaatcatcactgaggaaaaacatagatatctaatactgactggagtattagtcaaggcttatttcacacacaattttatcagaaaccaaagtagtttaaaacagctctccccttattagtaatgcattggagggtttactttaccatgtaccttgctgagcactgtaccttgttaatctcatttacttgtaatgagaaccacacagcgggtagttttattggttctattttacctacatgacaaaactgaagcataaaaacacttagtaagttttcagtgtcatgcacaactaggaagtgacatggccagaatataagcccagtcaccatcactctataacctgcgcttttaacaacttcagggcatgacacatttggccggtcagtagaacccatgctgtgatttgtttttgcagtggtggtgatgactgccttgttgaatccactttttattctattccattttggggacacaattctgcaagatgattcttcattaggaaacagagatgagttattgaccaacacagaaagaaaaagagtttgttgctccacactgggattaaacctatgatcttggcctaattaacactagctagtaagtgtccaagctgatcatctctacaacatttcaataacagaaaacaacaattttcaaaattagttacttacaattatgtagaaatgcctctaaaacacagtattttccttatattacaaaaacaaaaattataattggttttgtcctcttttgagagtttgcatggtgttactccctgcatagtgaagaaaacattttatttaagtagatggatctaagtttttcatgaacaaaggaatgacatttgaaatcaatcctaccctagtccaggagaatgcattagattaacctagtagaggtcttatttcaccctgagttttctatgatcgtgattctctgctggaggagtaattgtgaaatagatctctctgggaactggcttcctagtccaatcagctcttttaccaatgaacacttccttgtgatatagatgtttatggccgagaggatcctgggtaggaaacacatttgaatggtatttactaagatactaaaatccttggacttcactctaattttagtgccatttagaactcaaggtctcagtaaaagtagaaataaagcctgttaacaaaacacaaactgaatattaaaaatgtaactggattttcaaagaaatgtttactggtattacctgtagatgtatattctttattatgatcttttgtgtaaagtctggcagacaaatgcaatatctaattgttgagtccaatatcacaagcagtacaaaagtataaaaaagacttggccttttctaatgtgttaaaatactttatgctggtaataacactaagagtagggcactagaaattttaagtgaagataatgtgttgcagttactgcactcaatggcttactattataaaccaaaactgggatcactaagctccagtcagtcaaaatgatcaaaattattgaagagaataagcaattctgttctttattaggacacagtagatacagactacaaagtggagtgtgcttaataagaggtagcatttgttaagtgtcaattactctattatcccttggagcttctcaaaataaccatataaggtgtaagatgttaaaggttatggttacactcagtgcacaggtaagctaataggctgagagaagctaaattacttactggggtctcacagtaagaaagtgagctgaagtttcagcccagatttaactggattctgggctctttattcatgttacttcatgaatctgtttctcaattgtgcagaaaaaagggggctatttataagaaaagcaataaacaaacaagtaatgatctcaaataagtaatgcaagaaatagtgagatttcaaaatcagtggcagcgatttctcagttctgtcctaagtggccttgctcaatcacctgctatcttttagtggagctttgaaattatgtttcagacaacttcgattcagttctagaatgtttgactcagcaaattcacaggctcatctttctaacttgatggtgaatatggaaattcagctaaatggatgttaataaaattcaaacgttttaaggacagatggaaatgacagaattttaaggtaaaatatatgaaggaatataagataaaggatttttctaccttcagcaaaaacatacccactaattagtaaaattaataggcgaaaaaaagttgcatgctcttatactgtaatgattatcattttaaaactagctttttgccttcgagctatcggggtaaagacctacaggaaaactactgtcgaaatcctcgaggggaagaagggggaccctggtgtttcacaagcaatccagaggtacgctacgaagtctgtgacattcctcagtgttcagaagttgaatgcatgacctgcaatggggagagttatcgaggtctcatggatcatacagaatcaggcaagatttgtcagcgctgggatcatcagacaccacaccggcacaaattcttgcctgaaagatatcccgacaagggctttgatgataattattgccgcaatcccgatggccagccgaggccatggtgctatactcttgaccctcacacccgctgggagtactgtgcaattaaaacatgcgctgacaatactatgaatgacactgatgttcctttggaaacaactgaatgcatccaaggtcaaggagaaggctacaggggcactgtcaataccatttggaatggaattccatgtcagcgttgggattctcagtatcctcacgagcatgacatgactcctgaaaatttcaagtgcaaggacctacgagaaaattactgccgaaatccagatgggtctgaatcaccctggtgttttaccactgatccaaacatccgagttggctactgctcccaaattccaaactgtgatatgtcacatggacaagattgttatcgtgggaatggcaaaaattatatgggcaacttatcccaaacaagatctggactaacatgttcaatgtgggacaagaacatggaagacttacatcgtcatatcttctgggaaccagatgcaagtaagctgaatgagaattactgccgaaatccagatgatgatgctcatggaccctggtgctacacgggaaatccactcattccttgggattattgccctatttctcgttgtgaaggtgataccacacctacaatagtcaatttagaccatcccgtaatatcttgtgccaaaacgaaacaattgcgagttgtaaatgggattccaacacgaacaaacataggatggatggttagtttgagatacagaaataaacatatctgcggaggatcattgataaaggagagttgggttcttactgcacgacagtgtttcccttctcgagacttgaaagattatgaagcttggcttggaattcatgatgtccacggaagaggagatgagaaatgcaaacaggttctcaatgtttcccagctggtatatggccctgaaggatcagatctggttttaatgaagcttgccaggcctgctgtcctggatgattttgttagtacgattgatttacctaattatggatgcacaattcctgaaaagaccagttgcagtgtttatggctggggctacactggattgatcaactatgatggcctattacgagtggcacatctctatataatgggaaatgagaaatgcagccagcatcatcgagggaaggtgactctgaatgagtctgaaatatgtgctggggctgaaaagattggatcaggaccatgtgagggggattatggtggcccacttgtttgtgagcaacataaaatgagaatggttcttggtgtcattgttcctggtcgtggatgtgccattccaaatcgtcctggtatttttgtccgagtagcatattatgcaaaatggatacacaaaattattttaacatataaggtaccacagtcatag

SEQ ID NO: 10 - DNA, 4241 bp, synthetic construct
  source 1..4241: mol_type = other DNA
atgtgggtgaccaaactcctgccagccctgctgctgcagcatgtcctcctgcatctcctcctgctccccatcgccatcccctatgcagagggacaaaggaaaagaagaaatacaattcatgaattcaaaaaatcagcaaagactaccctaatcaaaatagatccagcactgaagataaaaaccaaaaaagtgaatactgcagaccaatgtgctaatagatgtactaggaataaaggacttccattcacttgcaaggcttttgtttttgataaagcaagaaaacaatgcctctggttccccttcaatagcatgtcaagtggagtgaaaaaagaatttggccatgaatttgacctctatgaaaacaaagactacattagaaactgcatcattggtaaaggacgcagctacaagggaacagtatctatcactaagagtggcatcaaatgtcagccctggagttccatgataccacacgaacacaggtaagaacagtatgaagaaaagagatgaagcctctgtcttttttacatgttaacagtctcatattagtccttcagaataattctacaatcctaaaataacttagccaacttgctgaattgtattacggcaaggtttatatgaattcatgactgatatttagcaaatgattaattaatatgttaataaaatgtagccaaaacaatatcttaccttaatgcctcaatttgtagatctcggtatttgtgaaataataacgtaaacttcgtttaaaaggattcttcttcctgtctttgagaaagtacggcactgtgcagggggagaggttgattgtgaaaaatcagaggtagatgagaatcttactgagggctgagggttctttaaccttggtggatctcaacattggttgcacattaaaatcacctgctgcaagcccttgacgaatcttacttagaagatgacaacacagaacaattaaatcagaatctctggggagaatagggcaccagtattttttgagctcccaccatgattccaaagtgcagccaaatttgagaaccactgctaaaagctcaagcttcagattgaccagcttttccatctcacctatcgcctaaagaccaaattggataaatgtgttcattacgacagatgggtactatttaaagatgagtaaacacaatatacttaggctcgtcagactgagagttttaatcatcactgaggaaaaacatagatatctaatactgactggagtattagtcaaggcttatttcacacacaattttatcagaaaccaaagtagtttaaaacagctctccccttattagtaatgcattggagggtttactttaccatgtaccttgctgagcactgtaccttgttaatctcatttacttgtaatgagaaccacacagcgggtagttttattggttctattttacctacatgacaaaactgaagcataaaaacacttagtaagttttcagtgtcatgcacaactaggaagtgacatggccagaatataagcccagtcaccatcactctataacctgcgcttttaacaacttcagggcatgacacatttggccggtcagtagaacccatgctgtgatttgtttttgcagtggtggtgatgactgccttgttgaatccactttttattctattccattttggggacacaattctgcaagatgattcttcattaggaaacagagatgagttattgaccaacacagaaagaaaaagagtttgttgctccacactgggattaaacctatgatcttggcctaattaacactagctagtaagtgtccaagctgatcatctctacaacatttcaataacagaaaacaacaattttcaaaattagttacttacaattatgtagaaatgcctctaaaacacagtattttccttatattacaaaaacaaaaattataattggttttgtcctcttttgagagtttgcatggtgttactccctgcatagtgaagaaaacattttatttaagtagatggatctaagtttttcatgaacaaaggaatgacatttgaaatcaatcctaccctagtccaggagaatgcattagattaacctagtagaggtcttatttcaccctgagttttctatgatcgtgattctctgctggaggagtaattgtgaaatagatctctctgggaactggcttcctagtccaatcagctcttttaccaatgaacacttccttgtgatatagatgtttatggccgagaggatccttatgtttcagacaacttcgattcagttctagaatgtttgactcagcaaattcacaggctcatctttctaacttgatggtgaatatggaaattcagctaaatggatgttaataaaattcaaacgttttaaggacagatggaaatgacagaattttaaggtaaaatatatgaaggaatataagataaaggatttttctaccttcagcaaaaacatacccactaattagtaaaattaataggcgaaaaaaagttgcatgctcttatactgtaatgattatcattttaaaactagctttttgccttcgagctatcggggtaaagacctacaggaaaactactgtcgaaatcctcgaggggaagaagggggaccctggtgtttcacaagcaatccagaggtacgctacgaagtctgtgacattcctcagtgttcagaagttgaatgcatgacctgcaatggggagagttatcgaggtctcatggatcatacagaatcaggcaagatttgtcagcgctgggatcatcagacaccacaccggcacaaattcttgcctgaaagatatcccgacaagggctttgatgataattattgccgcaatcccgatggccagccgaggccatggtgctatactcttgaccctcacacccgctgggagtactgtgcaattaaaacatgcgctgacaatactatgaatgacactgatgttcctttggaaacaactgaatgcatccaaggtcaaggagaaggctacaggggcactgtcaataccatttggaatggaattccatgtcagcgttgggattctcagtatcctcacgagcatgacatgactcctgaaaatttcaagtgcaaggacctacgagaaaattactgccgaaatccagatgggtctgaatcaccctggtgttttaccactgatccaaacatccgagttggctactgctcccaaattccaaactgtgatatgtcacatggacaagattgttatcgtgggaatggcaaaaattatatgggcaacttatcccaaacaagatctggactaacatgttcaatgtgggacaagaacatggaagacttacatcgtcatatcttctgggaaccagatgcaagtaagctgaatgagaattactgccgaaatccagatgatgatgctcatggaccctggtgctacacgggaaatccactcattccttgggattattgccctatttctcgttgtgaaggtgataccacacctacaatagtcaatttagaccatcccgtaatatcttgtgccaaaacgaaacaattgcgagttgtaaatgggattccaacacgaacaaacataggatggatggttagtttgagatacagaaataaacatatctgcggaggatcattgataaaggagagttgggttcttactgcacgacagtgtttcccttctcgagacttgaaagattatgaagcttggcttggaattcatgatgtccacggaagaggagatgagaaatgcaaacaggttctcaatgtttcccagctggtatatggccctgaaggatcagatctggttttaatgaagcttgccaggcctgctgtcctggatgattttgttagtacgattgatttacctaattatggatgcacaattcctgaaaagaccagttgcagtgtttatggctggggctacactggattgatcaactatgatggcctattacgagtggcacatctctatataatgggaaatgagaaatgcagccagcatcatcgagggaaggtgactctgaatgagtctgaaatatgtgctggggctgaaaagattggatcaggaccatgtgagggggattatggtggcccacttgtttgtgagcaacataaaatgagaatggttcttggtgtcattgttcctggtcgtggatgtgccattccaaatcgtcctggtatttttgtccgagtagcatattatgcaaaatggatacacaaaattattttaacatataaggtaccacagtcatag

SEQ ID NO: 11 - DNA, 5602 bp, synthetic construct
  source 1..5602: mol_type = other DNA
atgtgggtgaccaaactcctgccagccctgctgctgcagcatgtcctcctgcatctcctcctgctccccatcgccatcccctatgcagagggacaaaggaaaagaagaaatacaattcatgaattcaaaaaatcagcaaagactaccctaatcaaaatagatccagcactgaagataaaaaccaaaaaagtgaatactgcagaccaatgtgctaatagatgtactaggaataaaggacttccattcacttgcaaggcttttgtttttgataaagcaagaaaacaatgcctctggttccccttcaatagcatgtcaagtggagtgaaaaaagaatttggccatgaatttgacctctatgaaaacaaagactacattagaaactgcatcattggtaaaggacgcagctacaagggaacagtatctatcactaagagtggcatcaaatgtcagccctggagttccatgataccacacgaacacaggtaagaacagtatgaagaaaagagatgaagcctctgtcttttttacatgttaacagtctcatattagtccttcagaataattctacaatcctaaaataacttagccaacttgctgaattgtattacggcaaggtttatatgaattcatgactgatatttagcaaatgattaattaatatgttaataaaatgtagccaaaacaatatcttaccttaatgcctcaatttgtagatctcggtatttgtggatccagtatattaataaaatccctttttgtattcaatgagggaaacacataattttcatcaattagcagcttattggaatatctgcatgatggtttaacacttttaagtgttgactaaagattaattttacagaaaatagaaaaagaaatatgtttctgtctggaggaatgatttattgttgacccctaaattgaaatattttactagtggcttaatggaaagatgatgaaagatgatgaaattaatgtagaagcttaactagaaaatcaggtgacctgatatctacatctgtatccttcattggccacccagcattcattaatgaatcagatgatggaatagatcaagtttcctaggaacacagtgaatattaaaagaaaacaaagggagcctagcacctagaagacctagtttatatttcaaagtatatttggatgtaacccaattttaaacatttcctcacttgtctctcttaaagccttgccaacagcaaggacagagaaccaaaaatagtgtatatatgaataaatgcttattacagaatctgctgactggcacatgctttgtgtgtaatgggttctcataaacacttgttgaatgaacacacataagtgaaagagcatggctaggcttcatcccttggtcaaatatggggtgctaaagaaaagcaggggaaatacattgggacactaacaaaaaaaaacagttaatttaggtaaaagataaaatacaccacagaatgaagaaaagagatgacccagactgctctttaaccttcatgtcctagagaggtttttgatatgaattgcattcagaattgtggaaaggagcccatcttttctcttcattttgattttattaactccaatgggggaattttattcgtgttttggccatatctacttttgatttctacattattctctcttcctttctacctgtatttgtcctaataaattgttgacttattaattcactacttcctcacagcttttttttggctttacaaatccactggaaaggtatatgggtgtatcactttgtgtatttcggtgtgcatgtgtagaggggacaaaaatcctctctcaaactataaatattgagtatttgtgtattgaacatttgctataactactaggtttcttaaataatcttaatatataaaatgatatagaaaaagggaaattatagttcgtattattcatctaagtgaagagattaaaacccagggagtaaataaattgtctaaggactaaggttgtatactatttaggtgatagatatggggcaaccgtatgggttttatgattaacaaataaacttctcaccactctaccatatcaacttttccataaaagagagctatagtattctttgcttaaataaatttgattagtgcatgacttcttgaaaacatataaagcaaaagtcacatttgattctatcagaaaagtgagtaagccatggcccaaacaaaagatgcattaaaatattctggaatgatggagctaaaagtaagaaaaatgactttttaaaaaagtttactgttaggaattgtgaaattatgctgaattttagttgcattataatttttgtcagtcatacggtctgacaacctgtcttatttctatttccccatatgaggaatgctagttaagtatggatattaactattactacttagatgcattgaagttgcataatatggataatacttcactggttccctgaaaatgtttagttagtaataagtctcttacactatttgttttgtccaataatttatattttctgaagacttaactctagaatacactcatgtcaaaatgaaagaatttcattgcaaaatattgcttggtacatgacgcatacctgtatttgttttgtgtcacaacatgaaaaatgatggtttattagaagtttcattgggtaggaaacacatttgaatggtatttactaagatactaaaatccttggacttcactctaattttagtgccatttagaactcaaggtctcagtaaaagtagaaataaagcctgttaacaaaacacaaactgaatattaaaaatgtaactggattttcaaagaaatgtttactggtattacctgtagatgtatattctttattatgatcttttgtgtaaagtctggcagacaaatgcaatatctaattgttgagtccaatatcacaagcagtacaaaagtataaaaaagacttggccttttctaatgtgttaaaatactttatgctggtaataacactaagagtagggcactagaaattttaagtgaagataatgtgttgcagttactgcactcaatggcttactattataaaccaaaactgggatcactaagctccagtcagtcaaaatgatcaaaattattgaagagaataagcaattctgttctttattaggacacagtagatacagactacaaagtggagtgtgcttaataagaggtagcatttgttaagtgtcaattactctattatcccttggagcttctcaaaataaccatataaggtgtaagatgttaaaggttatggttacactcagtgcacaggtaagctaataggctgagagaagctaaattacttactggggtctcacagtaagaaagtgagctgaagtttcagcccagatttaactggattctgggctctttattcatgttacttcatgaatctgtttctcaattgtgcagaaaaaagggggctatttataagaaaagcaataaacaaacaagtaatgatctcaaataagtaatgcaagaaatagtgagatttcaaaatcagtggcagcgatttctcagttctgtcctaagtggccttgctcaatcacctgctatcttttagtggagctttgaaattatgtttcagacaacttcgattcagttctagaatgtttgactcagcaaattcacaggctcatctttctaacttgatggtgaatatggaaattcagctaaatggatgttaataaaattcaaacgttttaaggacagatggaaatgacagaattttaaggtaaaatatatgaaggaatataagataaaggatttttctaccttcagcaaaaacatacccactaattagtaaaattaataggcgaaaaaaagttgcatgctcttatactgtaatgattatcattttaaaactagctttttgccttcgagctatcggggtaaagacctacaggaaaactactgtcgaaatcctcgaggggaagaagggggaccctggtgtttcacaagcaatccagaggtacgctacgaagtctgtgacattcctcagtgttcagaagttgaatgcatgacctgcaatggggagagttatcgaggtctcatggatcatacagaatcaggcaagatttgtcagcgctgggatcatcagacaccacaccggcacaaattcttgcctgaaagatatcccgacaagggctttgatgataattattgccgcaatcccgatggccagccgaggccatggtgctatactcttgaccctcacacccgctgggagtactgtgcaattaaaacatgcgctgacaatactatgaatgacactgatgttcctttggaaacaactgaatgcatccaaggtcaaggagaaggctacaggggcactgtcaataccatttggaatggaattccatgtcagcgttgggattctcagtatcctcacgagcatgacatgactcctgaaaatttcaagtgcaaggacctacgagaaaattactgccgaaatccagatgggtctgaatcaccctggtgttttaccactgatccaaacatccgagttggctactgctcccaaattccaaactgtgatatgtcacatggacaagattgttatcgtgggaatggcaaaaattatatgggcaacttatcccaaacaagatctggactaacatgttcaatgtgggacaagaacatggaagacttacatcgtcatatcttctgggaaccagatgcaagtaagctgaatgagaattactgccgaaatccagatgatgatgctcatggaccctggtgctacacgggaaatccactcattccttgggattattgccctatttctcgttgtgaaggtgataccacacctacaatagtcaatttagaccatcccgtaatatcttgtgccaaaacgaaacaattgcgagttgtaaatgggattccaacacgaacaaacataggatggatggttagtttgagatacagaaataaacatatctgcggaggatcattgataaaggagagttgggttcttactgcacgacagtgtttcccttctcgagacttgaaagattatgaagcttggcttggaattcatgatgtccacggaagaggagatgagaaatgcaaacaggttctcaatgtttcccagctggtatatggccctgaaggatcagatctggttttaatgaagcttgccaggcctgctgtcctggatgattttgttagtacgattgatttacctaattatggatgcacaattcctgaaaagaccagttgcagtgtttatggctggggctacactggattgatcaactatgatggcctattacgagtggcacatctctatataatgggaaatgagaaatgcagccagcatcatcgagggaaggtgactctgaatgagtctgaaatatgtgctggggctgaaaagattggatcaggaccatgtgagggggattatggtggcccacttgtttgtgagcaacataaaatgagaatggttcttggtgtcattgttcctggtcgtggatgtgccattccaaatcgtcctggtatttttgtccgagtagcatattatgcaaaatggatacacaaaattattttaacatataaggtaccacagtcatag

SEQ ID NO: 12 - DNA, 4679 bp, synthetic construct
  source 1..4679: mol_type = other DNA
atgtgggtgaccaaactcctgccagccctgctgctgcagcatgtcctcctgcatctcctcctgctccccatcgccatcccctatgcagagggacaaaggaaaagaagaaatacaattcatgaattcaaaaaatcagcaaagactaccctaatcaaaatagatccagcactgaagataaaaaccaaaaaagtgaatactgcagaccaatgtgctaatagatgtactaggaataaaggacttccattcacttgcaaggcttttgtttttgataaagcaagaaaacaatgcctctggttccccttcaatagcatgtcaagtggagtgaaaaaagaatttggccatgaatttgacctctatgaaaacaaagactacattagaaactgcatcattggtaaaggacgcagctacaagggaacagtatctatcactaagagtggcatcaaatgtcagccctggagttccatgataccacacgaacacaggtaagaacagtatgaagaaaagagatgaagcctctgtcttttttacatgttaacagtctcatattagtccttcagaataattctacaatcctaaaataacttagccaacttgctgaattgtattacggcaaggtttatatgaattcatgactgatatttagcaaatgattaattaatatgttaataaaatgtagccaaaacaatatcttaccttaatgcctcaatttgtagatctcggtatttgtggatctcttcctttctacctgtatttgtcctaataaattgttgacttattaattcactacttcctcacagcttttttttggctttacaaatccactggaaaggtatatgggtgtatcactttgtgtatttcggtgtgcatgtgtagaggggacaaaaatcctctctcaaactataaatattgagtatttgtgtattgaacatttgctataactactaggtttcttaaataatcttaatatataaaatgatatagaaaaagggaaattatagttcgtattattcatctaagtgaagagattaaaacccagggagtaaataaattgtctaaggactaaggttgtatactatttaggtgatagatatggggcaaccgtatgggttttatgattaacaaataaacttctcaccactctaccatatcaacttttccataaaagagagctatagtattctttgcttaaataaatttgattagtgcatgacttcttgaaaacatataaagcaaaagtcacatttgattctatcagaaaagtgagtaagccatggcccaaacaaaagatgcattaaaatattctggaatgatggagctaaaagtaagaaaaatgactttttaaaaaagtttactgttaggaattgtgaaattatgctgaattttagttgcattataatttttgtcagtcatacggtctgacaacctgtcttatttctatttccccatatgaggaatgctagttaagtatggatattaactattactacttagatgcattgaagttgcataatatggataatacttcactggttccctgaaaatgtttagttagtaataagtctcttacactatttgttttgtccaataatttatattttctgaagacttaactctagaatacactcatgtcaaaatgaaagaatttcattgcaaaatattgcttggtacatgacgcatacctgtatttgttttgtgtcacaacatgaaaaatgatggtttattagaagtttcattgggtaggaaacacatttgaatggtatttactaagatactaaaatccttggacttcactctaattttagtgccatttagaactcaaggtctcagtaaaagtagaaataaagcctgttaacaaaacacaaactgaatattaaaaatgtaactggattttcaaagaaatgtttactggtattacctgtagatgtatattctttattatgatcttttgtgtaaagtctggcagacaaatgcaatatctaattgttgagtccaatatcacaagcagtacaaaagtataaaaaagacttggccttttctaatgtgttaaaatactttatgctggtaataacactaagagtagggcactagaaattttaagtgaagataatgtgttgcagttactgcactcaatggcttactattataaaccaaaactgggatcactaagctccagtcagtcaaaatgatcaaaattattgaagagaataagcaattctgttctttattaggacacagtagatacagactacaaagtggagtgtgcttaataagaggtagcatttgttaagtgtcaattactctattatcccttggagcttctcaaaataaccatataaggtgtaagatgttaaaggttatggttacactcagtgcacaggtaagctaataggctgagagaagctaaattacttactggggtctcacagtaagaaagtgagctgaagtttcagcccagatttaactggattctgggctctttattcatgttacttcatgaatctgtttctcaattgtgcagaaaaaagggggctatttataagaaaagcaataaacaaacaagtaatgatctcaaataagtaatgcaagaaatagtgagatttcaaaatcagtggcagcgatttctcagttctgtcctaagtggccttgctcaatcacctgctatcttttagtggagctttgaaattatgtttcagacaacttcgattcagttctagaatgtttgactcagcaaattcacaggctcatctttctaacttgatggtgaatatggaaattcagctaaatggatgttaataaaattcaaacgttttaaggacagatggaaatgacagaattttaaggtaaaatatatgaaggaatataagataaaggatttttctaccttcagcaaaaacatacccactaattagtaaaattaataggcgaaaaaaagttgcatgctcttatactgtaatgattatcattttaaaactagctttttgccttcgagctatcggggtaaagacctacaggaaaactactgtcgaaatcctcgaggggaagaagggggaccctggtgtttcacaagcaatccagaggtacgctacgaagtctgtgacattcctcagtgttcagaagttgaatgcatgacctgcaatggggagagttatcgaggtctcatggatcatacagaatcaggcaagatttgtcagcgctgggatcatcagacaccacaccggcacaaattcttgcctgaaagatatcccgacaagggctttgatgataattattgccgcaatcccgatggccagccgaggccatggtgctatactcttgaccctcacacccgctgggagtactgtgcaattaaaacatgcgctgacaatactatgaatgacactgatgttcctttggaaacaactgaatgcatccaaggtcaaggagaaggctacaggggcactgtcaataccatttggaatggaattccatgtcagcgttgggattctcagtatcctcacgagcatgacatgactcctgaaaatttcaagtgcaaggacctacgagaaaattactgccgaaatccagatgggtctgaatcaccctggtgttttaccactgatccaaacatccgagttggctactgctcccaaattccaaactgtgatatgtcacatggacaagattgttatcgtgggaatggcaaaaattatatgggcaacttatcccaaacaagatctggactaacatgttcaatgtgggacaagaacatggaagacttacatcgtcatatcttctgggaaccagatgcaagtaagctgaatgagaattactgccgaaatccagatgatgatgctcatggaccctggtgctacacgggaaatccactcattccttgggattattgccctatttctcgttgtgaaggtgataccacacctacaatagtcaatttagaccatcccgtaatatcttgtgccaaaacgaaacaattgcgagttgtaaatgggattccaacacgaacaaacataggatggatggttagtttgagatacagaaataaacatatctgcggaggatcattgataaaggagagttgggttcttactgcacgacagtgtttcccttctcgagacttgaaagattatgaagcttggcttggaattcatgatgtccacggaagaggagatgagaaatgcaaacaggttctcaatgtttcccagctggtatatggccctgaaggatcagatctggttttaatgaagcttgccaggcctgctgtcctggatgattttgttagtacgattgatttacctaattatggatgcacaattcctgaaaagaccagttgcagtgtttatggctggggctacactggattgatcaactatgatggcctattacgagtggcacatctctatataatgggaaatgagaaatgcagccagcatcatcgagggaaggtgactctgaatgagtctgaaatatgtgctggggctgaaaagattggatcaggaccatgtgagggggattatggtggcccacttgtttgtgagcaacataaaatgagaatggttcttggtgtcattgttcctggtcgtggatgtgccattccaaatcgtcctggtatttttgtccgagtagcatattatgcaaaatggatacacaaaattattttaacatataaggtaccacagtcatag

SEQ ID NO: 13 - DNA, 3679 bp, synthetic construct
  source 1..3679: mol_type = other DNA
atgtgggtgaccaaactcctgccagccctgctgctgcagcatgtcctcctgcatctcctcctgctccccatcgccatcccctatgcagagggacaaaggaaaagaagaaatacaattcatgaattcaaaaaatcagcaaagactaccctaatcaaaatagatccagcactgaagataaaaaccaaaaaagtgaatactgcagaccaatgtgctaatagatgtactaggaataaaggacttccattcacttgcaaggcttttgtttttgataaagcaagaaaacaatgcctctggttccccttcaatagcatgtcaagtggagtgaaaaaagaatttggccatgaatttgacctctatgaaaacaaagactacattagaaactgcatcattggtaaaggacgcagctacaagggaacagtatctatcactaagagtggcatcaaatgtcagccctggagttccatgataccacacgaacacaggtaagaacagtatgaagaaaagagatgaagcctctgtcttttttacatgttaacagtctcatattagtccttcagaataattctacaatcctaaaataacttagccaacttgctgaattgtattacggcaaggtttatatgaattcatgactgatatttagcaaatgattaattaatatgttaataaaatgtagccaaaacaatatcttaccttaatgcctcaatttgtagatctcggtatttgtggatcctgggtaggaaacacatttgaatggtatttactaagatactaaaatccttggacttcactctaattttagtgccatttagaactcaaggtctcagtaaaagtagaaataaagcctgttaacaaaacacaaactgaatattaaaaatgtaactggattttcaaagaaatgtttactggtattacctgtagatgtatattctttattatgatcttttgtgtaaagtctggcagacaaatgcaatatctaattgttgagtccaatatcacaagcagtacaaaagtataaaaaagacttggccttttctaatgtgttaaaatactttatgctggtaataacactaagagtagggcactagaaattttaagtgaagataatgtgttgcagttactgcactcaatggcttactattataaaccaaaactgggatcactaagctccagtcagtcaaaatgatcaaaattattgaagagaataagcaattctgttctttattaggacacagtagatacagactacaaagtggagtgtgcttaataagaggtagcatttgttaagtgtcaattactctattatcccttggagcttctcaaaataaccatataaggtgtaagatgttaaaggttatggttacactcagtgcacaggtaagctaataggctgagagaagctaaattacttactggggtctcacagtaagaaagtgagctgaagtttcagcccagatttaactggattctgggctctttattcatgttacttcatgaatctgtttctcaattgtgcagaaaaaagggggctatttataagaaaagcaataaacaaacaagtaatgatctcaaataagtaatgcaagaaatagtgagatttcaaaatcagtggcagcgatttctcagttctgtcctaagtggccttgctcaatcacctgctatcttttagtggagctttgaaattatgtttcagacaacttcgattcagttctagaatgtttgactcagcaaattcacaggctcatctttctaacttgatggtgaatatggaaattcagctaaatggatgttaataaaattcaaacgttttaaggacagatggaaatgacagaattttaaggtaaaatatatgaaggaatataagataaaggatttttctaccttcagcaaaaacatacccactaattagtaaaattaataggcgaaaaaaagttgcatgctcttatactgtaatgattatcattttaaaactagctttttgccttcgagctatcggggtaaagacctacaggaaaactactgtcgaaatcctcgaggggaagaagggggaccctggtgtttcacaagcaatccagaggtacgctacgaagtctgtgacattcctcagtgttcagaagttgaatgcatgacctgcaatggggagagttatcgaggtctcatggatcatacagaatcaggcaagatttgtcagcgctgggatcatcagacaccacaccggcacaaattcttgcctgaaagatatcccgacaagggctttgatgataattattgccgcaatcccgatggccagccgaggccatggtgctatactcttgaccctcacacccgctgggagtactgtgcaattaaaacatgcgctgacaatactatgaatgacactgatgttcctttggaaacaactgaatgcatccaaggtcaaggagaaggctacaggggcactgtcaataccatttggaatggaattccatgtcagcgttgggattctcagtatcctcacgagcatgacatgactcctgaaaatttcaagtgcaaggacctacgagaaaattactgccgaaatccagatgggtctgaatcaccctggtgttttaccactgatccaaacatccgagttggctactgctcccaaattccaaactgtgatatgtcacatggacaagattgttatcgtgggaatggcaaaaattatatgggcaacttatcccaaacaagatctggactaacatgttcaatgtgggacaagaacatggaagacttacatcgtcatatcttctgggaaccagatgcaagtaagctgaatgagaattactgccgaaatccagatgatgatgctcatggaccctggtgctacacgggaaatccactcattccttgggattattgccctatttctcgttgtgaaggtgataccacacctacaatagtcaatttagaccatcccgtaatatcttgtgccaaaacgaaacaattgcgagttgtaaatgggattccaacacgaacaaacataggatggatggttagtttgagatacagaaataaacatatctgcggaggatcattgataaaggagagttgggttcttactgcacgacagtgtttcccttctcgagacttgaaagattatgaagcttggcttggaattcatgatgtccacggaagaggagatgagaaatgcaaacaggttctcaatgtttcccagctggtatatggccctgaaggatcagatctggttttaatgaagcttgccaggcctgctgtcctggatgattttgttagtacgattgatttacctaattatggatgcacaattcctgaaaagaccagttgcagtgtttatggctggggctacactggattgatcaactatgatggcctattacgagtggcacatctctatataatgggaaatgagaaatgcagccagcatcatcgagggaaggtgactctgaatgagtctgaaatatgtgctggggctgaaaagattggatcaggaccatgtgagggggattatggtggcccacttgtttgtgagcaacataaaatgagaatggttcttggtgtcattgttcctggtcgtggatgtgccattccaaatcgtcctggtatttttgtccgagtagcatattatgcaaaatggatacacaaaattattttaacatataaggtaccacagtcatag

SEQ ID NO: 14 - DNA, 2730 bp, synthetic construct
  source 1..2730: mol_type = other DNA
atgtgggtgaccaaactcctgccagccctgctgctgcagcatgtcctcctgcatctcctcctgctccccatcgccatcccctatgcagagggacaaaggaaaagaagaaatacaattcatgaattcaaaaaatcagcaaagactaccctaatcaaaatagatccagcactgaagataaaaaccaaaaaagtgaatactgcagaccaatgtgctaatagatgtactaggaataaaggacttccattcacttgcaaggcttttgtttttgataaagcaagaaaacaatgcctctggttccccttcaatagcatgtcaagtggagtgaaaaaagaatttggccatgaatttgacctctatgaaaacaaagactacattagaaactgcatcattggtaaaggacgcagctacaagggaacagtatctatcactaagagtggcatcaaatgtcagccctggagttccatgataccacacgaacacaggtaagaacagtatgaagaaaagagatgaagcctctgtcttttttacatgttaacagtctcatattagtccttcagaataattctacaatcctaaaataacttagccaacttgctgaattgtattacggcaaggtttatatgaattcatgactgatatttagcaaatgattaattaatatgttaataaaatgtagccaaaacaatatcttaccttaatgcctcaatttgtagatctcggtatttgtggatccttatgtttcagacaacttcgattcagttctagaatgtttgactcagcaaattcacaggctcatctttctaacttgatggtgaatatggaaattcagctaaatggatgttaataaaattcaaacgttttaaggacagatggaaatgacagaattttaaggtaaaatatatgaaggaatataagataaaggatttttctaccttcagcaaaaacatacccactaattagtaaaattaataggcgaaaaaaagttgcatgctcttatactgtaatgattatcattttaaaactagctttttgccttcgagctatcggggtaaagacctacaggaaaactactgtcgaaatcctcgaggggaagaagggggaccctggtgtttcacaagcaatccagaggtacgctacgaagtctgtgacattcctcagtgttcagaagttgaatgcatgacctgcaatggggagagttatcgaggtctcatggatcatacagaatcaggcaagatttgtcagcgctgggatcatcagacaccacaccggcacaaattcttgcctgaaagatatcccgacaagggctttgatgataattattgccgcaatcccgatggccagccgaggccatggtgctatactcttgaccctcacacccgctgggagtactgtgcaattaaaacatgcgctgacaatactatgaatgacactgatgttcctttggaaacaactgaatgcatccaaggtcaaggagaaggctacaggggcactgtcaataccatttggaatggaattccatgtcagcgttgggattctcagtatcctcacgagcatgacatgactcctgaaaatttcaagtgcaaggacctacgagaaaattactgccgaaatccagatgggtctgaatcaccctggtgttttaccactgatccaaacatccgagttggctactgctcccaaattccaaactgtgatatgtcacatggacaagattgttatcgtgggaatggcaaaaattatatgggcaacttatcccaaacaagatctggactaacatgttcaatgtgggacaagaacatggaagacttacatcgtcatatcttctgggaaccagatgcaagtaagctgaatgagaattactgccgaaatccagatgatgatgctcatggaccctggtgctacacgggaaatccactcattccttgggattattgccctatttctcgttgtgaaggtgataccacacctacaatagtcaatttagaccatcccgtaatatcttgtgccaaaacgaaacaattgcgagttgtaaatgggattccaacacgaacaaacataggatggatggttagtttgagatacagaaataaacatatctgcggaggatcattgataaaggagagttgggttcttactgcacgacagtgtttcccttctcgagacttgaaagattatgaagcttggcttggaattcatgatgtccacggaagaggagatgagaaatgcaaacaggttctcaatgtttcccagctggtatatggccctgaaggatcagatctggttttaatgaagcttgccaggcctgctgtcctggatgattttgttagtacgattgatttacctaattatggatgcacaattcctgaaaagaccagttgcagtgtttatggctggggctacactggattgatcaactatgatggcctattacgagtggcacatctctatataatgggaaatgagaaatgcagccagcatcatcgagggaaggtgactctgaatgagtctgaaatatgtgctggggctgaaaagattggatcaggaccatgtgagggggattatggtggcccacttgtttgtgagcaacataaaatgagaatggttcttggtgtcattgttcctggtcgtggatgtgccattccaaatcgtcctggtatttttgtccgagtagcatattatgcaaaatggatacacaaaattattttaacatataaggtaccacagtcatag

SEQ ID NO: 15 - DNA, 3250 bp, synthetic construct
  source 1..3250: mol_type = other DNA
cagggtcggaacaggagagcgcacgagggagcttccagggggaaacgcctggtatctttatagtcctgtcgggtttcgccacctctgacttgagcgtcgatttttgtgatgctcgtcaggggggcggagcctatggaaaaacgccagcaacgcggcctttttacggttcctggccttttgctggccttttgctcacatgcgcgttgacattgattattgactagttattaatagtaatcaattacggggtcattagttcatagcccatatatggagttccgcgttacataacttacggtaaatggcccgcctggctgaccgcccaacgacccccgcccattgacgtcaataatgacgtatgttcccatagtaacgccaatagggactttccattgacgtcaatgggtggagtatttacggtaaactgcccacttggcagtacatcaagtgtatcatatgccaagtccgccccctattgacgtcaatgacggtaaatggcccgcctggcattatgcccagtacatgaccttacgggactttcctacttggcagtacatctacgtattagtcatcgctattaccatggtgatgcggttttggcagtacaccaatgggcgtggatagcggtttgactcacggggatttccaagtctccaccccattgacgtcaatgggagtttgttttggcaccaaaatcaacgggactttccaaaatgtcgtaataaccccgccccgttgacgcaaatgggcggtaggcgtgtacggtgggaggtctatataagcagagctcgtttagtgaaccgtcagatcgcctggagacgccatccacgctgttttgacctccatagaagacaccgggaccgatccagcctccgcggccgggaacggtgcattggaacgcggattccccgtgccaagagtgacgtaagtaccgcctatagactctataggcacacccctttggctcttatgcatgctatactgtttttggcttggggcctatacacccccgcttccttatgctataggtgatggtatagcttagcctataggtgtgggttattgaccattattgaccactcccctattggtgacgatactttccattactaatccataacatggctctagacttaaggcagcggcagaagaagatgtaggcagctgagttgttgtattctgataagagtcagaggtaactcccgttgcggtgctgttaacggtggagggcagtgtagtctgagcagtactcgttgctgccgcgcgcgccaccagacataatagctgacagactaacagactgttcctttccatgggtcttttctgcagtcaccgtccttgacacgaagcttatcgatgtcgacctcgagtctagagggcccgtttaaacccgctgatcagcctcgactgtgccttctagttgccagccatctgttgtttgcccctcccccgtgccttccttgaccctggaaggtgccactcccactgtcctttcctaataaaatgaggaaattgcatcgcattgtctgagtaggtgtcattctattctggggggtggggtggggcaggacagcaagggggaggattgggaagacaatagcaggcatgctggggagtcgaaattcagaagaactcgtcaagaaggcgatagaaggcgatgcgctgcgaatcgggagcggcgataccgtaaagcacgaggaagcggtcagcccattcgccgccaagctcttcagcaatatcacgggtagccaacgctatgtcctgatagcggtccgccacacccagccggccacagtcgatgaatccagaaaagcggccattttccaccatgatattcggcaagcaggcatcgccatgggtcacgacgagatcctcgccgtcgggcatgctcgccttgagcctggcgaacagttcggctggcgcgagcccctgatgctcttcgtccagatcatcctgatcgacaagaccggcttccatccgagtacgtgctcgctcgatgcgatgtttcgcttggtggtcgaatgggcaggtagccggatcaagcgtatgcagccgccgcattgcatcagccatgatggatactttctcggcaggagcaaggtgagatgacaggagatcctgccccggcacttcgcccaatagcagccagtcccttcccgcttcagtgacaacgtcgagcacagctgcgcaaggaacgcccgtcgtggccagccacgatagccgcgctgcctcgtcttgcagttcattcagggcaccggacaggtcggtcttgacaaaaagaaccgggcgcccctgcgctgacagccggaacacggcggcatcagagcagccgattgtctgttgtgcccagtcatagccgaatagcctctccacccaagcggccggagaacctgcgtgcaatccatcttgttcaatcatgcgaaacgatcctcatcctgtctcttgatcagatcttgatcccctgcgccatcagatccttggcggcaagaaagccatccagtttactttgcagggcttcccaaccttaccagagggcgccccagctggcaattccggttcgcttgctgcgtcagaccccgtagaaaagatcaaaggatcttcttgagatcctttttttctgcgcgtaatctgctgcttgcaaacaaaaaaaccaccgctaccagcggtggtttgtttgccggatcaagagctaccaactctttttccgaaggtaactggcttcagcagagcgcagataccaaatactgttcttctagtgtagccgtagttaggccaccacttcaagaactctgtagcaccgcctacatacctcgctctgctaatcctgttaccagtggctgctgccagtggcgataagtcgtgtcttaccgggttggactcaagacgatagttaccggataaggcgcagcggtcgggctgaacggggggttcgtgcacacagcccagcttggagcgaacgacctacaccgaactgagatacctacagcgtgagctatgagaaagcgccacgcttcccgaagggagaaaggcggacaggtatccggtaagcggcagggtcggaacaggagagcgcacgagggagcttccagggggaaacgcctggtatctttatagtcctgtcgggtttcgccacctctgacttgagcgtcgatttttgtgatgctcgtcaggggggcggagcctatggaaaaacgccagcaacgcggcctttttacggttcctggccttttgctggccttttgctcacatg

SEQ ID NO: 16 - DNA, 858 bp, Homo sapiens
  source 1..858: mol_type = other DNA
atgggaaaaatcagcagtcttccaacccaattatttaagtgctgcttttgtgatttcttgaaggtgaagatgcacaccatgtcctcctcgcatctcttctacctggcgctgtgcctgctcaccttcaccagctctgccacggctggaccggagacgctctgcggggctgagctggtggatgctcttcagttcgtgtgtggagacaggggcttttatttcaacaagcccacagggtatggctccagcagtcggagggcgcctcagacaggcatcgtggatgagtgctgcttccggagctgtgatctaaggaggctggagatgtattgcgcacccctcaagcctgccaagtcagctcgctctgtccgtgcccagcgccacaccgacatgcccaagacccagaaggtaagcccacctgggtgggatccagccatcctcaagtggtctctctcttgtgcatgtgggtgggccaagcagaaatcctgccccatagtctcctggcttacaagtcagaaaagctcctttgcaccaaagggatggattacatccccatctctttgctaaacaaacatgggctttggtgtcagacaaaagtgaagtcctggctttctcacacaccagcttagagagaaaagacttttaggtgaatgtggcaggaaagcgtgcttgctggggcaaaggcagattcattctttctcttcccagtatcagcccccatctaccaacaagaacacgaagtctcagagaaggaaaggaagtacatttgaagaacgcaagtagctttttctcctttatttataggaagtacatttgaagaacgcaagtagagggagtgcaggaaacaagaactacaggatgtag

SEQ ID NO: 17 - DNA, 270 bp, Homo sapiens
  source 1..270: mol_type = other DNA
atgaacgccaaggtcgtggtcgtgctggtcctcgtgctgaccgcgctctgcctcagcgacgggaagcccgtcagcctgagctacagatgcccatgccgattcttcgaaagccatgttgccagagccaacgtcaagcatctcaaaattctcaacactccaaactgtgcccttcagattgtagcccggctgaagaacaacaacagacaagtgtgcattgacccgaagctaaagtggattcaggagtacctggagaaagctttaaacaagtaa

SEQ ID NO: 18 - DNA, 4173 bp, Homo sapiens
  source 1..4173: mol_type = other DNA
atgaaggcccccgctgtgcttgcacctggcatcctcgtgctcctgtttaccttggtgcagaggagcaatggggagtgtaaagaggcactagcaaagtccgagatgaatgtgaatatgaagtatcagcttcccaacttcaccgcggaaacacccatccagaatgtcattctacatgagcatcacattttccttggtgccactaactacatttatgttttaaatgaggaagaccttcagaaggttgctgagtacaagactgggcctgtgctggaacacccagattgtttcccatgtcaggactgcagcagcaaagccaatttatcaggaggtgtttggaaagataacatcaacatggctctagttgtcgacacctactatgatgatcaactcattagctgtggcagcgtcaacagagggacctgccagcgacatgtctttccccacaatcatactgctgacatacagtcggaggttcactgcatattctccccacagatagaagagcccagccagtgtcctgactgtgtggtgagcgccctgggagccaaagtcctttcatctgtaaaggaccggttcatcaacttctttgtaggcaataccataaattcttcttatttcccagatcatccattgcattcgatatcagtgagaaggctaaaggaaacgaaagatggttttatgtttttgacggaccagtcctacattgatgttttacctgagttcagagattcttaccccattaagtatgtccatgcctttgaaagcaacaattttatttacttcttgacggtccaaagggaaactctagatgctcagacttttcacacaagaataatcaggttctgttccataaactctggattgcattcctacatggaaatgcctctggagtgtattctcacagaaaagagaaaaaagagatccacaaagaaggaagtgtttaatatacttcaggctgcgtatgtcagcaagcctggggcccagcttgctagacaaataggagccagcctgaatgatgacattcttttcggggtgttcgcacaaagcaagccagattctgccgaaccaatggatcgatctgccatgtgtgcattccctatcaaatatgtcaacgacttcttcaacaagatcgtcaacaaaaacaatgtgagatgtctccagcatttttacggacccaatcatgagcactgctttaataggacacttctgagaaattcatcaggctgtgaagcgcgccgtgatgaatatcgaacagagtttaccacagctttgcagcgcgttgacttattcatgggtcaattcagcgaagtcctcttaacatctatatccaccttcattaaaggagacctcaccatagctaatcttgggacatcagagggtcgcttcatgcaggttgtggtttctcgatcaggaccatcaacccctcatgtgaattttctcctggactcccatccagtgtctccagaagtgattgtggagcatacattaaaccaaaatggctacacactggttatcactgggaagaagatcacgaagatcccattgaatggcttgggctgcagacatttccagtcctgcagtcaatgcctctctgccccaccctttgttcagtgtggctggtgccacgacaaatgtgtgcgatcggaggaatgcctgagcgggacatggactcaacagatctgtctgcctgcaatctacaaggttttcccaaatagtgcaccccttgaaggagggacaaggctgaccatatgtggctgggactttggatttcggaggaataataaatttgatttaaagaaaactagagttctccttggaaatgagagctgcaccttgactttaagtgagagcacgatgaatacattgaaatgcacagttggtcctgccatgaataagcatttcaatatgtccataattatttcaaatggccacgggacaacacaatacagtacattctcctatgtggatcctgtaataacaagtatttcgccgaaatacggtcctatggctggtggcactttacttactttaactggaaattacctaaacagtgggaattctagacacatttcaattggtggaaaaacatgtactttaaaaagtgtgtcaaacagtattcttgaatgttataccccagcccaaaccatttcaactgagtttgctgttaaattgaaaattgacttagccaaccgagagacaagcatcttcagttaccgtgaagatcccattgtctatgaaattcatccaaccaaatcttttattagtggtgggagcacaataacaggtgttgggaaaaacctgaattcagttagtgtcccgagaatggtcataaatgtgcatgaagcaggaaggaactttacagtggcatgtcaacatcgctctaattcagagataatctgttgtaccactccttccctgcaacagctgaatctgcaactccccctgaaaaccaaagcctttttcatgttagatgggatcctttccaaatactttgatctcatttatgtacataatcctgtgtttaagccttttgaaaagccagtgatgatctcaatgggcaatgaaaatgtactggaaattaagggaaatgatattgaccctgaagcagttaaaggtgaagtgttaaaagttggaaataagagctgtgagaatatacacttacattctgaagccgttttatgcacggtccccaatgacctgctgaaattgaacagcgagctaaatatagagtggaagcaagcaatttcttcaaccgtccttggaaaagtaatagttcaaccagatcagaatttcacaggattgattgctggtgttgtctcaatatcaacagcactgttattactacttgggtttttcctgtggctgaaaaagagaaagcaaattaaagatctgggcagtgaattagttcgctacgatgcaagagtacacactcctcatttggataggcttgtaagtgcccgaagtgtaagcccaactacagaaatggtttcaaatgaatctgtagactaccgagctacttttccagaagatcagtttcctaattcatctcagaacggttcatgccgacaagtgcagtatcctctgacagacatgtcccccatcctaactagtggggactctgatatatccagtccattactgcaaaatactgtccacattgacctcagtgctctaaatccagagctggtccaggcagtgcagcatgtagtgattgggcccagtagcctgattgtgcatttcaatgaagtcataggaagagggcattttggttgtgtatatcatgggactttgttggacaatgatggcaagaaaattcactgtgctgtgaaatccttgaacagaatcactgacataggagaagtttcccaatttctgaccgagggaatcatcatgaaagattttagtcatcccaatgtcctctcgctcctgggaatctgcctgcgaagtgaagggtctccgctggtggtcctaccatacatgaaacatggagatcttcgaaatttcattcgaaatgagactcataatccaactgtaaaagatcttattggctttggtcttcaagtagccaaaggcatgaaatatcttgcaagcaaaaagtttgtccacagagacttggctgcaagaaactgtatgctggatgaaaaattcacagtcaaggttgctgattttggtcttgccagagacatgtatgataaagaatactatagtgtacacaacaaaacaggtgcaaagctgccagtgaagtggatggctttggaaagtctgcaaactcaaaagtttaccaccaagtcagatgtgtggtcctttggcgtgctcctctgggagctgatgacaagaggagccccaccttatcctgacgtaaacacctttgatataactgtttacttgttgcaagggagaagactcctacaacccgaatactgcccagaccccttatatgaagtaatgctaaaatgctggcaccctaaagccgaaatgcgcccatccttttctgaactggtgtcccggatatcagcgatcttctctactttcattggggagcactatgtccatgtgaacgctacttatgtgaacgtaaaatgtgtcgctccgtatccttctctgttgtcatcagaagataacgctgatgatgaggtggacacacgaccagcctccttctgggagacatcatag

SEQ ID NO: 19 - protein, 137 aa, Homo sapiens
MITPTVKMHTMSSSHLFYLALCLLTFTSSATAGPETLCGAELVDALQFVCGDRGFYFNKPTGYGSSSRRAPQTGIVDECCFRSCDLRRLEMYCAPLKPAKSARSVRAQRHTDMPKTQKEVHLKNASRGSAGNKNYRM

SEQ ID NO: 20 - protein, 158 aa, Homo sapiens
MGKISSLPTQLFKCCFCDFLKVKMHTMSSSHLFYLALCLLTFTSSATAGPETLCGAELVDALQFVCGDRGFYFNKPTGYGSSSRRAPQTGIVDECCFRSCDLRRLEMYCAPLKPAKSARSVRAQRHTDMPKTQKYQPPSTNKNTKSQRRKGSTFEERK

SEQ ID NO: 21 - protein, 89 aa, Homo sapiens
MNAKVVVVLVLVLTALCLSDGKPVSLSYRCPCRFFESHVARANVKHLKILNTPNCALQIVARLKNNNRQVCIDPKLKWIQEYLEKALNK

SEQ ID NO: 22 - protein, 68 aa, Homo sapiens
KPVSLSYRCPCRFFESHVARANVKHLKILNTPNCALQIVARLKNNNRQVCIDPKLKWIQEYLEKALNK